European Patent Specification EP 3 684 404 B1, published June 24, 2026. Title: Immunogenic Chikungunya Virus. Applicant: Valneva SE. The sequence listing filed with the application follows.

SEQUENCE LISTING (49 sequences)

SEQ ID NO: 1 - DNA, 11674 bp, Chikungunya virus
gatggctgcgtgagacacacgtagcctaccagtttcttactgctctactctgcaaagcaagagattaataacccatcatggatcctgtgtacgtggacatagacgctgacagcgcctttttgaaggccctgcaacgtgcgtaccccatgtttgaggtggaaccaaggcaggtcacaccgaatgaccatgctaatgctagagcgttctcgcatctagctataaaactaatagagcaggaaattgaccccgactcaaccatcctggatatcggcagtgcgccagcaaggaggatgatgtcggacaggaagtaccactgcgtctgcccgatgcgcagtgcggaagatcccgagagactcgccaattatgcgagaaagctagcatctgccgcaggaaaagtcctggacagaaacatctctggaaagatcggggacttacaagcagtaatggccgtgccagacacggagacgccaacattctgcttacacacagacgtctcatgtagacagagagcagacgtcgctatataccaagacgtctatgctgtacacgcacccacgtcgctataccaccaggcgattaaaggggtccgagtggcgtactgggttgggttcgacacaaccccgttcatgtacaatgccatggcgggtgcctacccctcatactcgacaaactgggcagatgagcaggtactgaaggctaagaacataggattatgttcaacagacctgacggaaggtagacgaggcaagttgtctattatgagagggaaaaagctaaaaccgtgcgaccgtgtgctgttctcagtagggtcaacgctctacccggaaagccgcaagctacttaagagctggcacctgccatcggtgttccatttaaagggcaaactcagcttcacatgccgctgtgatacagtggtttcgtgtgagggctacgtcgttaagagaataacgatgagcccaggcctttatggaaaaaccacagggtatgcggtaacccaccacgcagacggattcctgatgtgcaagactaccgacacggttgacggcgaaagaatgtcattctcggtgtgcacatacgtgccggcgaccatttgtgatcaaatgaccggcatccttgctacagaagtcacgccggaggatgcacagaagctgttggtggggctgaaccagagaatagtggttaacggcagaacgcaacggaatacgaacaccatgaaaaattatctgcttcccgtggtcgcccaagccttcagtaagtgggcaaaggagtgccggaaagacatggaagatgaaaaactcctgggggtcagagaaagaacactgacctgctgctgtctatgggcattcaagaagcagaaaacacacacggtctacaagaggcctgatacccagtcaattcagaaggttcaggccgagtttgacagctttgtggtaccgagtctgtggtcgtccgggttgtcaatccctttgaggactagaatcaaatggttgttaagcaaggtgccaaaaaccgacctgatcccatacagcggagacgcccgagaagcccgggacgcagaaaaagaagcagaggaagaacgagaagcagaactgactcgcgaagccctaccacctctacaggcagcacaggaagatgttcaggtcgaaatcgacgtggaacagcttgaggacagagcgggcgcaggaataatagagactccgagaggagctatcaaagttactgcccaaccaacagaccacgtcgtgggagagtacctggtactctccccgcagaccgtactacgtagccagaagctcagtctgattcacgctttggcggagcaagtgaagacgtgcacgcacaacggacgagcagggaggtatgcggtcgaagcgtacgacggccgagtcctagtgccctcaggctatgcaatctcgcctgaagacttccagagtctaagcgaaagcgcaacgatggtgtataacgaaagagagttcgtaaacagaaagctacaccatattgcgatgcacggaccagccctgaacaccgacgaagagtcgtatgagctggtgagggcagagaggacagaacacgagtacgtctacgacgtggatcagagaagatgctgtaagaaggaagaagccgcaggactggtactggtgggcgacttgactaatccgccctaccacgaattcgcatatgaagggctaaaaatccgccctgcctgcccatacaaaattgcagtcataggagtcttcggagtaccgggatctggcaagtcagctattatcaagaacctagttaccaggcaggacctggtgactagcggaaagaaagaaaactgccaagaaatcaccaccgacgtgatgagacagagaggtctagagatatctgcacgtacggttgactcgctgctcttgaatggatgcaacagaccagtcgacgtgttgtacgtagacgaggcgtttgcgtgccactctggaacgctacttgctttgatcgccttggtgagaccaaggcagaaagttgtactttgtggtgacccgaagcagtgcggcttcttcaatatgatgcagatgaaagtcaactataatcacaacatctgcacccaagtgtaccacaaaagtatctccaggcggtgtacactgcctgtgaccgccattgtgtcatcgttgcattacgaaggcaaaatgcgcactacgaatgagtacaacaagccgattgtagtggacactacaggctcaacaaaacctgaccctggagacctcgtgttaacgtgcttcagagggtgggttaaacaactgcaaattgactatcgtggatacgaggtcatgacagcagccgcatcccaagggttaaccagaaaaggagtttacgcagttagacaaaaagttaatgaaaacccgctctatgcatcaacgtcagagcacgtcaacgtactcctaacgcgtacggaaggtaaactggtatggaagacactttccggcgacccgtggataaagacgctgcagaacccaccgaaaggaaacttcaaagcaactattaaggagtgggaggtggagcatgcatcaataatggcgggcatctgcagtcaccaaatgaccttcgatacattccaaaataaagccaacgtttgttgggctaagagcttggtccctatcctcgaaacagcggggataaaactaaatgataggcagtggtctcagataattcaagccttcaaagaagacaaagcatactcacctgaagtagccctgaatgaaatatgtacgcgcatgtatggggtggatctagacagcgggctattttctaaaccgttggtgtctgtgtattacgcggataaccactgggataataggcctggagggaaaatgttcggatttaaccccgaggcagcatccattctagaaagaaagtatccattcacaaaagggaagtggaacatcaacaagcagatctgcgtgactaccaggaggatagaagactttaaccctaccaccaacatcataccggccaacaggagactaccacactcattagtggccgaacaccgcccagtaaaaggggaaagaatggaatggctggttaacaagataaacggccaccacgtgctcctggtcagtggctataaccttgcactgcctactaagagagtcacttgggtagcgccgttaggtgtccgcggagcggactacacatacaacctagagttgggtctgccagcaacgcttggtaggtatgacctagtggtcataaacatccacacaccttttcgcatacaccattaccaacagtgcgtcgaccacgcaatgaaactgcaaatgctcgggggtgactcattgagactgctcaaaccgggcggctctctattgatcagagcatatggttacgcagatagaaccagtgaacgagtcatctgcgtattgggacgcaagtttagatcgtctagagcgttgaaaccaccatgtgtcaccagcaacactgagatgtttttcctattcagcaactttgacaatggcagaaggaatttcacaactcatgtcatgaacaatcaactgaatgcagccttcgtaggacaggtcacccgagcaggatgtgcaccgtcgtaccgggtaaaacgcatggacatcgcgaagaacgatgaagagtgcgtagtcaacgccgctaaccctcgcgggttaccgggtggcggtgtttgcaaggcagtatacaaaaaatggccggagtcctttaagaacagtgcaacaccagtgggaaccgcaaaaacagttatgtgcggtacgtatccagtaatccacgctgttggaccaaacttctctaattattcggagtctgaaggggaccgggaattggcagctgcctatcgagaagtcgcaaaggaagtaactaggctgggagtaaatagtgtagctatacctctcctctccacaggtgtatactcaggagggaaagacaggctgacccagtcactgaaccacctctttacagccatggactcgacggatgcagacgtggtcatctactgccgcgacaaagaatgggagaagaaaatatctgaggccatacagatgcggacccaagtagagctgctggatgagcacatctccatagactgcgatattgttcgcgtgcaccctgacagcagcttggcaggcagaaaaggatacagcaccacggaaggcgcactgtactcatatctagaagggacccgttttcatcagacggctgtggatatggcggagatacatactatgtggccaaagcaaacagaggccaatgagcaagtctgcctatatgccctgggggaaagtattgaatcgatcaggcagaaatgcccggtggatgatgcagacgcatcatctccccccaaaactgtcccgtgcctttgccgttacgctatgactccagaacgcgtcacccggcttcgcatgaaccacgtcacaagcataattgtgtgttcttcgtttcccctcccaaagtacaaaatagaaggagtgcaaaaagtcaaatgctctaaggtaatgctatttgaccacaacgtgccatcgcgcgtaagtccaagggcttatagaggtgccgctgccggtaaccttgcggccgtgtctgattgggtaatgagcaccgtacctgtcgcgccgcccagaagaaggcgagggagaaacctgactgtgacatgtgacgagagagaagggaatataacacccatggctagcgtccgattctttagggcagagctgtgtccggtcgtacaagaaacagcggagacgcgtgacacagcaatgtctcttcaggcaccaccgagtaccgccacggaaccgaatcatccgccgatctccttcggagcatcaagcgagacgttccccattacatttggggacttcaacgaaggagaaatcgaaagcttgtcttctgagctactaactttcggagacttcttaccaggagaagtggatgacttgacagacagcgactggtccacgtgctcagacacggacgacgagttaagactagacagggcaggtgggtatatattctcgtcggacaccggtccaggtcatttacaacagaagtcagtacgccagtcagtgctgccggtgaacaccctggaggaagtccacgaggagaagtgttacccacctaagctggatgaagcaaaggagcaactattacttaagaaactccaggagagtgcatccatggccaacagaagcaggtatcagtcgcgcaaagtagaaaacatgaaagcagcaatcatccagagactaaagagaggctgtagactatacttaatgtcagagaccccaaaagtccctacttaccggactacatatccggcgcctgtgtactcgcctccgatcaacgtccgattgtccaatcccgagtccgcagtggcagcatgcaatgagttcttagctagaaactatccaactgtctcatcataccaaattaccgacgagtatgatgcatatctagacatggtggacgggtcggagagttgcctggaccgagcgacattcaatccgtcaaaactcaggagctacccgaaacagcacgcttaccacgcgccctccatcagaagcgctgtaccgtccccattccagaacacactacagaatgtactggcagcagccacgaaaagaaactgcaacgtcacacagatgagggaattacccactttggactcagcagtattcaacgtggagtgtttcaaaaaattcgcatgcaaccaagaatactgggaagaatttgctgccagccctattaggataacaactgagaatttagcaacctatgttactaaactaaaagggccaaaagcagcagcgctattcgcaaaaacccataatctactgccactacaggaagtaccaatggataggttcacagtagatatgaaaagggacgtaaaggtgactcctggtacaaagcatacagaggaaagacctaaggtgcaggttatacaggcggctgaacccttggcgacagcatacctatgtgggattcacagagagctggttaggaggctgaacgccgtcctcctacccaatgtacatacactatttgacatgtctgccgaggatttcgatgccatcatagccgcacactttaagccaggagacactgttttggaaacggacatagcctcctttgataagagccaagatgattcacttgcgcttactgctttgatgctgttagaggatttaggggtggatcactccctgctggacttgatagaggctgctttcggagagatttccagctgtcacctaccgacaggtacgcgcttcaagttcggcgccatgatgaaatcaggtatgttcctaactctgttcgtcaacacattgttaaacatcaccatcgccagccgagtgctggaagatcgtctgacaaaatccgcgtgcgcggccttcatcggcgacgacaacataatacatggagtcgtctccgatgaattgatggcagccagatgtgccacttggatgaacatggaagtgaagatcatagatgcagttgtatccttgaaagccccttacttttgtggagggtttatactgcacgatactgtgacaggaacagcttgcagagtggcagacccgctaaaaaggctttttaaactgggcaaaccgctagcggcaggtgacgaacaagatgaagatagaagacgagcgctggctgacgaagtgatcagatggcaacgaacagggctaattgatgagctggagaaagcggtatactctaggtacgaagtgcagggtatatcagttgtggtaatgtccatggccacctttgcaagctccagatccaacttcgagaagctcagaggacccgtcataactttgtacggcggtcctaaataggtacgcactacagctacctattttgcagaagccgacagcaagtatctaaacactaatcagctacaatggagttcatcccaacccaaactttttacaataggaggtaccagcctcgaccctggactccgcgccctactatccaagtcatcaggcccagaccgcgccctcagaggcaagctgggcaacttgcccagctgatctcagcagttaataaactgacaatgcgcgcggtaccacaacagaagccacgcaggaatcggaagaataagaagcaaaagcaaaaacaacaggcgccacaaaacaacacaaatcaaaagaagcagccacctaaaaagaaaccggctcaaaagaaaaagaagccgggccgcagagagaggatgtgcatgaaaatcgaaaatgattgtattttcgaagtcaagcacgaaggtaaggtaacaggttacgcgtgcctggtgggggacaaagtaatgaaaccagcacacgtaaaggggaccatcgataacgcggacctggccaaactggcctttaagcggtcatctaagtatgaccttgaatgcgcgcagatacccgtgcacatgaagtccgacgcttcgaagttcacccatgagaaaccggaggggtactacaactggcaccacggagcagtacagtactcaggaggccggttcaccatccctacaggtgctggcaaaccaggggacagcggcagaccgatcttcgacaacaagggacgcgtggtggccatagtcttaggaggagctaatgaaggagcccgtacagccctctcggtggtgacctggaataaagacattgtcactaaaatcacccccgagggggccgaagagtggagtcttgccatcccagttatgtgcctgttggcaaacaccacgttcccctgctcccagcccccttgcacgccctgctgctacgaaaaggaaccggaggaaaccctacgcatgcttgaggacaacgtcatgagacctgggtactatcagctgctacaagcatccttaacatgttctccccaccgccagcgacgcagcaccaaggacaacttcaatgtctataaagccacaagaccatacttagctcactgtcccgactgtggagaagggcactcgtgccatagtcccgtagcactagaacgcatcagaaatgaagcgacagacgggacgctgaaaatccaggtctccttgcaaatcggaataaagacggatgacagccacgattggaccaagctgcgttatatggacaaccacatgccagcagacgcagagagggcggggctatttgtaagaacatcagcaccgtgtacgattactggaacaatgggacacttcatcctggcccgatgtccaaaaggggaaactctgacggtgggattcactgacagtaggaagattagtcactcatgtacgcacccatttcaccacgaccctcctgtgataggtcgggaaaaattccattcccgaccgcagcacggtaaagagctaccttgcagcacgtacgtgcagagcaccgccgcaactaccgaggagatagaggtacacatgcccccagacacccctgatcgcacattaatgtcacaacagtccggcaacgtaaagatcacagtcaatggccagacggtgcggtacaagtgtaattgcggtggctcaaatgaaggactaacaactacagacaaagtgattaataactgcaaggttgatcaatgtcatgccgcggtcaccaatcacaaaaagtggcagtataactcccctctggtcccgcgtaatgctgaacttggggaccgaaaaggaaaaattcacatcccgtttccgctggcaaatgtaacatgcagggtgcctaaagcaaggaaccccaccgtgacgtacgggaaaaaccaagtcatcatgctactgtatcctgaccacccaacactcctgtcctaccggaatatgggagaagaaccaaactatcaagaagagtgggtgatgcataagaaggaagtcgtgctaaccgtgccgactgaagggctcgaggtcacgtggggcaacaacgagccgtataagtattggccgcagttatctacaaacggtacagcccatggccacccgcatgagataattctgtattattatgagctgtaccccactatgactgtagtagttgtgtcagtggccacgttcatactcctgtcgatggtgggtatggcagcggggatgtgcatgtgtgcacgacgcagatgcatcacaccgtatgaactgacaccaggagctaccgtccctttcctgcttagcctaatatgctgcatcagaacagctaaagcggccacataccaagaggctgcgatatacctgtggaacgagcagcaacctttgttttggctacaagcccttattccgctggcagccctgattgttctatgcaactgtctgagactcttaccatgctgctgtaaaacgttggcttttttagccgtaatgagcgtcggtgcccacactgtgagcgcgtacgaacacgtaacagtgatcccgaacacggtgggagtaccgtataagactctagtcaatagacctggctacagccccatggtattggagatggaactactgtcagtcactttggagccaacactatcgcttgattacatcacgtgcgagtacaaaaccgtcatcccgtctccgtacgtgaagtgctgcggtacagcagagtgcaaggacaaaaacctacctgactacagctgtaaggtcttcaccggcgtctacccatttatgtggggcggcgcctactgcttctgcgacgctgaaaacacgcagttgagcgaagcacacgtggagaagtccgaatcatgcaaaacagaatttgcatcagcatacagggctcataccgcatctgcatcagctaagctccgcgtcctttaccaaggaaataacatcactgtaactgcctatgcaaacggcgaccatgccgtcacagttaaggacgccaaattcattgtggggccaatgtcttcagcctggacacctttcgacaacaaaattgtggtgtacaaaggtgacgtctataacatggactacccgccctttggcgcaggaagaccaggacaatttggcgatatccaaagtcgcacacctgagagtaaagacgtctatgctaatacacaactggtactgcagagaccggctgtgggtacggtacacgtgccatactctcaggcaccatctggctttaagtattggctaaaagaacgcggggcgtcgctgcagcacacagcaccatttggctgccaaatagcaacaaacccggtaagagcggtgaactgcgccgtagggaacatgcccatctccatcgacataccggaagcggccttcactagggtcgtcgacgcgccctctttaacggacatgtcgtgcgaggtaccagcctgcacccattcctcagactttgggggcgtcgccattattaaatatgcagccagcaagaaaggcaagtgtgcggtgcattcgatgactaacgccgtcactattcgggaagctgagatagaagttgaagggaattctcagctgcaaatctctttctcgacggccttagccagcgccgaattccgcgtacaagtctgttctacacaagtacactgtgcagccgagtgccaccccccgaaggaccacatagtcaactacccggcgtcacataccaccctcggggtccaggacatctccgctacggcgatgtcatgggtgcagaagatcacgggaggtgtgggactggttgttgctgttgccgcactgattctaatcgtggtgctatgcgtgtcgttcagcaggcactaacttgacaattaagtatgaaggtatatgtgtcccctaagagacacactgtacatagcaaataatctatagatcaaagggctacgcaacccctgaatagtaacaaaatacaaaatcactaaaaattataaaaacagaaaaatacataaataggtatacgtgtcccctaagagacacattgtatgtaggtgataagtatagatcaaagggccgaataacccctgaatagtaacaaaatatgaaaatcaataaaaatcataaaatagaaaaaccataaacagaagtagttcaaagggctataaaacccctgaatagtaacaaaacataaaattaataaaaatcaaatgaataccataattggcaaacggaagagatgtaggtacttaagcttcctaaaagcagccgaactcactttgagaagtaggcatagcataccgaactcttccacgattctccgaacccacagggacgtaggagatgttattttgtttttaatatttcaaaaaaaaaaaaaaaaaaaaaaaa

SEQ ID NO: 2 - protein, 423 aa, Chikungunya virus
STKDNFNVYKATRPYLAHCPDCGEGHSCHSPVALERIRNEATDGTLKIQVSLQIGIKTDDSHDWTKLRYMDNHMPADAERAGLFVRTSAPCTITGTMGHFILARCPKGETLTVGFTDSRKISHSCTHPFHHDPPVIGREKFHSRPQHGKELPCSTYVQSTAATTEEIEVHMPPDTPDHTLMSQQSGNVKITVNGQTVRYKCNCGGSNEGLTTTDKVINNCKVDQCHAAVTNHKKWQYNSPLVPRNAELGDRKGKIHIPFPLANVTCRVPKARNPTVTYGKNQVIMLLYPDHPTLLSYRNMGEEPNYQEEWVMHKKEVVLTVPTEGLEVTWGNNEPYKYWPQLSTNGTAHGHPHEIILYYYELYPTMTVVVVSVATFILLSMVGMAAGMCMCARRRCITPYELTPGATVPFLLSLICCIRTAKA

SEQ ID NO: 3 - protein, 423 aa, Artificial Sequence
  mutation arising from Vero passaging
STKDNFNVYKATRPYLAHCPDCGEGHSCHSPVALERIRNEATDGTLKIQVSLQIGIKTDDSHDWTKLRYMDNHMPADAERAGLFVRTSAPCTITGTMGHFILARCPKGETLTVGFTDSRKISHSCTHPFHHDPPVIGREKFHSRPQHGKELPCSTYVQSTAATTEEIKVHMPPDTPDHTLMSQQSGNVKITVNGQTVRYKCNCGGSNEGLTTTDKVINNCKVDQCHAAVTNHKKWQYNSPLVPRNAELGDRKGKIHIPFPLANVTCRVPKARNPTVTYGKNQVIMLLYPDHPTLLSYRNMGEEPNYQEEWVMHKKEVVLTVPTEGLEVTWGNNEPYKYWPQLSTNGTAHGHPHEIILYYYELYPTMTVVVVSVATFILLSMVGMAAGMCMCARRRCITPYELTPGATVPFLLSLICCIRTAKA

SEQ ID NO: 4 - protein, 423 aa, Artificial Sequence
  mutation arising from Vero passaging
STKDNFNVYKATRPYLAHCPDCGEGHSCHSPVALERIRNEATDGTLKIQVSLQIRIKTDDSHDWTKLRYMDNHMPADAERAGLFVRTSAPCTITGTMGHFILARCPKGETLTVGFTDSRKISHSCTHPFHHDPPVIGREKFHSRPQHGKELPCSTYVQSTAATTEEIEVHMPPDTPDHTLMSQQSGNVKITVNGQTVRYKCNCGGSNEGLTTTDKVINNCKVDQCHAAVTNHKKWQYNSPLVPRNAELGDRKGKIHIPFPLANVTCRVPKARNPTVTYGKNQVIMLLYPDHPTLLSYRNMGEEPNYQEEWVMHKKEVVLTVPTEGLEVTWGNNEPYKYWPQLSTNGTAHGHPHEIILYYYELYPTMTVVVVSVATFILLSMVGMAAGMCMCARRRCITPYELTPGATVPFLLSLICCIRTAKA

SEQ ID NO: 5 - protein, 423 aa, Artificial Sequence
  mutation arising from Vero passaging
STKDNFNVYKATRPYLAHCPDCGEGHSCHSPVALERIRNEATDGTLKIQVSLQIGIKTDDSHDWTKLRYMDNHMPADAERAGLFVRTSAPCTITGTMGHFILARCPKGETLTVGFTDSRKISHSCTHPFHHDPPVIGREKFHSRPQHGKELPCSTYVQSTAATTEEIEVHMPPDTPDHTLMSQQSGNVKITVNGQTVRYKCNCGGSNEGLTTTDKVINNCKVDQCHAAVTNHKKWQYNSPLVPRNAKLGDRKGKIHIPFPLANVTCRVPKARNPTVTYGKNQVIMLLYPDHPTLLSYRNMGEEPNYQEEWVMHKKEVVLTVPTEGLEVTWGNNEPYKYWPQLSTNGTAHGHPHEIILYYYELYPTMTVVVVSVATFILLSMVGMAAGMCMCARRRCITPYELTPGATVPFLLSLICCIRTAKA

SEQ ID NO: 6 - protein, 423 aa, Artificial Sequence
  mutation arising from Vero passaging
STKDNFNVYKATRPYLAHCPDCGEGHSCHSPVALERIRNEATDGTLKIQVSLQIGIKTDDSHDWTKLRYMDNHMPADAERARLFVRTSAPCTITGTMGHFILARCPKGETLTVGFTDSRKISHSCTHPFHHDPPVIGREKFHSRPQHGKELPCSTYVQSTAATTEEIEVHMPPDTPDHTLMSQQSGNVKITVNGQTVRYKCNCGGSNEGLTTTDKVINNCKVDQCHAAVTNHKKWQYNSPLVPRNAELGDRKGKIHIPFPLANVTCRVPKARNPTVTYGKNQVIMLLYPDHPTLLSYRNMGEEPNYQEEWVMHKKEVVLTVPTEGLEVTWGNNEPYKYWPQLSTNGTAHGHPHEIILYYYELYPTMTVVVVSVATFILLSMVGMAAGMCMCARRRCITPYELTPGATVPFLLSLICCIRTAKA

SEQ ID NO: 7 - protein, 423 aa, Artificial Sequence
  mutation arising from Vero passaging
STKDNFNVYKATRPYLAHCPDCGEGHSCHSPVALERIRNEATDGTLKIQVSLQIGIKTDDSHDWTKLRYMDNHMPADAERAGLFVRTSAPCTITGTMGHFILARCPKGETLTVGFTDSRKISHSCTHPFHHDPPVIGREKFHSRPQHGKELPCSTYVQSTAATTEEIEVHMPPDTPDHTLMSQQSGNVKITVNGQTVRYKCNCGGSNEGLTTTDKVINNCKVDQCHAAVTNYKKWQYNSPLVPRNAELGDRKGKIHIPFPLANVTCRVPKARNPTVTYGKNQVIMLLYPDHPTLLSYRNMGEEPNYQEEWVMHKKEVVLTVPTEGLEVTWGNNEPYKYWPQLSTNGTAHGHPHEIILYYYELYPTMTVVVVSVATFILLSMVGMAAGMCMCARRRCITPYELTPGATVPFLLSLICCIRTAKA

SEQ ID NO: 8 - DNA, 27 bp, Artificial Sequence
  primer
ttaggatccgatggctgcgtgagacac

SEQ ID NO: 9 - DNA, 29 bp, Artificial Sequence
  primer
taactcgagccgtcaggtctgttgaacat

SEQ ID NO: 10 - DNA, 28 bp, Artificial Sequence
  primer
ttaggatcctaccaccaggcgattaaag

SEQ ID NO: 11 - DNA, 29 bp, Artificial Sequence
  primer
taactcgagctttgcccacttactgaagg

SEQ ID NO: 12 - DNA, 27 bp, Artificial Sequence
  primer
ttaggatcctgctacagaagtcacgcc

SEQ ID NO: 13 - DNA, 26 bp, Artificial Sequence
  primer
taactcgaggccaaagcgtgaatcag

SEQ ID NO: 14 - DNA, 29 bp, Artificial Sequence
  primer
ttaggatccaacagcttgaggacagagcg

SEQ ID NO: 15 - DNA, 28 bp, Artificial Sequence
  primer
taactcgagctctgtctcatcacgtcgg

SEQ ID NO: 16 - DNA, 32 bp, Artificial Sequence
  primer
ttaggatccaaattgcagtcataggagtcttc

SEQ ID NO: 17 - DNA, 29 bp, Artificial Sequence
  primer
taactcgagagtacgttgacgtgctctga

SEQ ID NO: 18 - DNA, 29 bp, Artificial Sequence
  primer
ttaggatccgtgggttaaacaactgcaaa

SEQ ID NO: 19 - DNA, 33 bp, Artificial Sequence
  primer
taactcgagggttaaagtcttctatcctcctgg

SEQ ID NO: 20 - DNA, 31 bp, Artificial Sequence
  primer
ttaggatccggataaccactgggataatagg

SEQ ID NO: 21 - DNA, 30 bp, Artificial Sequence
  primer
taactcgagagttgtgaaattccttctgcc

SEQ ID NO: 22 - DNA, 29 bp, Artificial Sequence
  primer
ttaggatcccgcagatagaaccagtgaac

SEQ ID NO: 23 - DNA, 28 bp, Artificial Sequence
  primer
taactcgagcagcagctctacttgggtc

SEQ ID NO: 24 - DNA, 27 bp, Artificial Sequence
  primer
ttaggatccaggagggaaagacaggct

SEQ ID NO: 25 - DNA, 25 bp, Artificial Sequence
  primer
taactcgagccctcgccttcttctg

SEQ ID NO: 26 - DNA, 32 bp, Artificial Sequence
  primer
ttaggatcccaaaatagaaggagtgcaaaaag

SEQ ID NO: 27 - DNA, 35 bp, Artificial Sequence
  primer
taactcgagcctggagtttcttaagtaatagttgc

SEQ ID NO: 28 - DNA, 27 bp, Artificial Sequence
  primer
ttaggatccaccggtccaggtcattta

SEQ ID NO: 29 - DNA, 27 bp, Artificial Sequence
  primer
taactcgaggcagcaaattcttcccag

SEQ ID NO: 30 - DNA, 30 bp, Artificial Sequence
  primer
ttaggatccccattccagaacacactacag

SEQ ID NO: 31 - DNA, 29 bp, Artificial Sequence
  primer
taactcgagatacctgatttcatcatggc

SEQ ID NO: 32 - DNA, 30 bp, Artificial Sequence
  primer
ttaggatcccctttgataagagccaagatg

SEQ ID NO: 33 - DNA, 30 bp, Artificial Sequence
  primer
taactcgagtacaaagttatgacgggtcct

SEQ ID NO: 34 - DNA, 28 bp, Artificial Sequence
  primer
ttaggatcccaacgaacagggctaattg

SEQ ID NO: 35 - DNA, 26 bp, Artificial Sequence
  primer
taactcgaggaccgcttaaaggccag

SEQ ID NO: 36 - DNA, 29 bp, Artificial Sequence
  primer
ttaggatccgtgcatgaaaatcgaaaatg

SEQ ID NO: 37 - DNA, 31 bp, Artificial Sequence
  primer
taactcgagtggtcttgtggctttatagaca

SEQ ID NO: 38 - DNA, 27 bp, Artificial Sequence
  primer
ttaggatccaaccggaggaaaccctac

SEQ ID NO: 39 - DNA, 25 bp, Artificial Sequence
  primer
taactcgaggtaccgcaccgtctgg

SEQ ID NO: 40 - DNA, 27 bp, Artificial Sequence
  primer
ttaggatccagctaccttgcagcacgt

SEQ ID NO: 41 - DNA, 24 bp, Artificial Sequence
  primer
taactcgagcccaccatcgacagg

SEQ ID NO: 42 - DNA, 29 bp, Artificial Sequence
  primer
ttaggatcccgagccgtataagtattggc

SEQ ID NO: 43 - DNA, 27 bp, Artificial Sequence
  primer
taactcgagcgccggtgaagaccttac

SEQ ID NO: 44 - DNA, 32 bp, Artificial Sequence
  primer
ttaggatccactactgtcagtcactttggagc

SEQ ID NO: 45 - DNA, 29 bp, Artificial Sequence
  primer
taactcgagtaccgggtttgttgctattt

SEQ ID NO: 46 - DNA, 30 bp, Artificial Sequence
  primer
ttaggatcccacaactggtactgcagagac

SEQ ID NO: 47 - DNA, 30 bp, Artificial Sequence
  primer
taactcgaggcgtagccctttgatctatag

SEQ ID NO: 48 - DNA, 26 bp, Artificial Sequence
  primer
ttaggatccggtgctatgcgtgtcgt

SEQ ID NO: 49 - DNA, 29 bp, Artificial Sequence
  primer
taactcgagatctcctacgtccctgtggg